European Patent Application EP 4 420 526 A1, published August 28, 2024. Title: Composition for Preventing or Treating Muscular disease containing Ponciri Fructus extract. Applicant: KOREA INSTITUTE OF SCIENCE AND TECHNOLOGY. Application EP. The sequence listing filed with the application follows.

SEQUENCE LISTING (18 sequences)

SEQ ID NO: 1 - DNA, 20 bp, synthetic construct
  misc_feature 1..20: note = Myf5_primer F
  source 1..20: mol_type = other DNA
tccaggtattcccacctgct

SEQ ID NO: 2 - DNA, 24 bp, synthetic construct
  misc_feature 1..24: note = Myf5_primer R
  source 1..24: mol_type = other DNA
cacctggagcggatgaagaagaac

SEQ ID NO: 3 - DNA, 20 bp, synthetic construct
  misc_feature 1..20: note = Myf6_primer F
  source 1..20: mol_type = other DNA
acagatcgtcggaaagcagc

SEQ ID NO: 4 - DNA, 20 bp, synthetic construct
  misc_feature 1..20: note = Myf6_primer R
  source 1..20: mol_type = other DNA
cactccgcagaatctccacc

SEQ ID NO: 5 - DNA, 20 bp, synthetic construct
  misc_feature 1..20: note = Myod_primer F
  source 1..20: mol_type = other DNA
catagacttgacaggccccg

SEQ ID NO: 6 - DNA, 20 bp, synthetic construct
  misc_feature 1..20: note = Myod_primer R
  source 1..20: mol_type = other DNA
cgggtccaggtcctcaaaaa

SEQ ID NO: 7 - DNA, 20 bp, synthetic construct
  misc_feature 1..20: note = Myog_primer F
  source 1..20: mol_type = other DNA
agctatccggttccaaagcc

SEQ ID NO: 8 - DNA, 20 bp, synthetic construct
  misc_feature 1..20: note = Myog_primer R
  source 1..20: mol_type = other DNA
gcacaggagaccttggtcag

SEQ ID NO: 9 - DNA, 20 bp, synthetic construct
  misc_feature 1..20: note = Ppard_primer F
  source 1..20: mol_type = other DNA
gtatgcgcatgggactcact

SEQ ID NO: 10 - DNA, 20 bp, synthetic construct
  misc_feature 1..20: note = Ppard_primer R
  source 1..20: mol_type = other DNA
actgcctttaccgtgggttt

SEQ ID NO: 11 - DNA, 20 bp, synthetic construct
  misc_feature 1..20: note = Ppargc1a_primer F
  source 1..20: mol_type = other DNA
gttgcctgcatgagtgtgtg

SEQ ID NO: 12 - DNA, 20 bp, synthetic construct
  misc_feature 1..20: note = Ppargc1a_primer R
  source 1..20: mol_type = other DNA
cacatgtcccaagccatcca

SEQ ID NO: 13 - DNA, 20 bp, synthetic construct
  misc_feature 1..20: note = Ucp3_primer F
  source 1..20: mol_type = other DNA
gttttgcggacctcctcact

SEQ ID NO: 14 - DNA, 20 bp, synthetic construct
  misc_feature 1..20: note = Ucp3_primer R
  source 1..20: mol_type = other DNA
ctctgtgcgcaccatagtca

SEQ ID NO: 15 - DNA, 20 bp, synthetic construct
  misc_feature 1..20: note = Nrf1_primer F
  source 1..20: mol_type = other DNA
cccgtgttcctttgtggtga

SEQ ID NO: 16 - DNA, 20 bp, synthetic construct
  misc_feature 1..20: note = Nrf1_primer R
  source 1..20: mol_type = other DNA
attccatgctctgctgctgg

SEQ ID NO: 17 - DNA, 20 bp, synthetic construct
  misc_feature 1..20: note = Tomm20_primer F
  source 1..20: mol_type = other DNA
tgtgcggtgtgttgtctgtt

SEQ ID NO: 18 - DNA, 20 bp, synthetic construct
  misc_feature 1..20: note = Tomm20_primer R
  source 1..20: mol_type = other DNA
taagtgcccagagcacagga